European Patent Specification EP 3 377 102 B1, published August 9, 2023. Title: ANTI-PD-1 ANTIBODIES AND THERAPEUTIC USES THEREOF. Applicant: Lyvgen Biopharma. Application Not Yet Assigned. The sequence listing filed with the application follows.

SEQUENCE LISTING (24 sequences)

SEQ ID NO: 1 - protein, 107 aa, Artificial Sequence
  Synthetic Polypeptide
NIQMTQSPSLLSASVGDRVTLSCKAGQNVNNYLAWYQQKLGEPPKVLIFNANSLQTGVPSRFSGSGSGTDFTLTISSLQPEDVATYFCQQYNSWTTFGAGTKLELKR

SEQ ID NO: 2 - protein, 95 aa, Artificial Sequence
  Synthetic Polypeptide
DIQMTQSPSSLSASVGDRVTITCRASQGISNYLAWFQQKPGKAPKSLIYAASSLQSGVPSRFSGSGSGTDFTLTISSLQPEDFATYYCQQYNSYP

SEQ ID NO: 3 - protein, 12 aa, Artificial Sequence
  Synthetic Polypeptide
LTFGGGTKVEIK

SEQ ID NO: 4 - protein, 121 aa, Artificial Sequence
  Synthetic Polypeptide
QVTLKESGPGILQPSQTLSLTCSFSGFSLSTSGTCVSWIRQPSGKGLEWLATICWEDSKGYNPSLKNRLTISKDTSNNQAFLKITSVDTADSAIYYCARREDSGYFWFPYWGQGTLVSVSS

SEQ ID NO: 5 - protein, 100 aa, Artificial Sequence
  Synthetic Polypeptide
QVTLKESGPALVKPTQTLTLTCTFSGFSLSTSGMRVSWIRQPPGKALEWLARIDWDDDKFYSTSLKTRLTISKDTSKNQVVLTMTNMDPVDTATYYCARI

SEQ ID NO: 6 - protein, 15 aa, Artificial Sequence
  Synthetic Polypeptide
YFDYWGQGTLVTVSS

SEQ ID NO: 7 - protein, 107 aa, Artificial Sequence
  Synthetic Polypeptide
NIQMTQSPSSLSASVGDRVTITCKAGQNVNNYLAWYQQKPGKAPKVLIFNANSLQTGVPSRFSGSGSGTDFTLTISSLQPEDFATYYCQQYNSWTTFGGGTKVEIKR

SEQ ID NO: 8 - protein, 107 aa, Rattus rattus; identical to SEQ ID NO: 1

SEQ ID NO: 9 - protein, 121 aa, Artificial Sequence
  Synthetic Polypeptide
QVTLKESGPALVKPTQTLTLTCTFSGFSLSTSGTCVSWIRQPPGKALEWLATICWEDSKGYNPSLKSRLTISKDTSKNQAVLTMTNMDPVDTATYYCARREDSGYFWFPYWGQGTLVTVSS

SEQ ID NO: 10 - protein, 121 aa, Rattus rattus; identical to SEQ ID NO: 4

SEQ ID NO: 11 - protein, 107 aa, Artificial Sequence; identical to SEQ ID NO: 7
  Synthetic Polypeptide

SEQ ID NO: 12 - protein, 121 aa, Artificial Sequence; identical to SEQ ID NO: 9
  Synthetic Polypeptide

SEQ ID NO: 13 - protein, 9 aa, Artificial Sequence
  Synthetic Polypeptide
GFSLSTSGT

SEQ ID NO: 14 - protein, 5 aa, Artificial Sequence
  Synthetic Polypeptide
CWEDS

SEQ ID NO: 15 - protein, 10 aa, Artificial Sequence
  Synthetic Polypeptide
EDSGYFWFPY

SEQ ID NO: 16 - protein, 11 aa, Artificial Sequence
  Synthetic Polypeptide
KAGQNVNNYLA

SEQ ID NO: 17 - protein, 7 aa, Artificial Sequence
  Synthetic Polypeptide
NANSLQT

SEQ ID NO: 18 - protein, 8 aa, Artificial Sequence
  Synthetic Polypeptide
QQYNSWTT

SEQ ID NO: 19 - protein, 448 aa, Artificial Sequence
  Synthetic Polypeptide
QVTLKESGPGILQPSQTLSLTCSFSGFSLSTSGTCVSWIRQPSGKGLEWLATICWEDSKGYNPSLKNRLTISKDTSNNQAFLKITSVDTADSAIYYCARREDSGYFWFPYWGQGTLVSVSSASTKGPSVFPLAPCSRSTSESTAALGCLVKDYFPEPVTVSWNSGALTSGVHTFPAVLQSSGLYSLSSVVTVPSSSLGTKTYTCNVDHKPSNTKVDKRVESKYGPPCPPCPAPEFLGGPSVFLFPPKPKDTLMISRTPEVTCVVVDVSQEDPEVQFNWYVDGVEVHNAKTKPREEQFNSTYRVVSVLTVLHQDWLNGKEYKCKVSNKGLPSSIEKTISKAKGQPREPQVYTLPPSQEEMTKNQVSLTCLVKGFYPSDIAVEWESNGQPENNYKTTPPVLDSDGSFFLYSRLTVDKSRWQEGNVFSCSVMHEALHNHYTQKSLSLSLGK

SEQ ID NO: 20 - DNA, 1347 bp, Artificial Sequence
  Synthetic Polynucleotide
caggtgacactcaaggaaagcggacctggaatcctccaaccttcccagactctttccctgacctgtagcttctccgggttctccttgtccacctctggcacatgcgtgtcatggatcagacagccatctgggaagggcttggagtggctggcaacaatttgctgggaggattcaaaggggtacaaccccagtctgaagaacaggctgaccattagcaaggacaccagcaacaatcaggccttcctgaaaattactagcgtcgatacagctgacagcgccatctactactgcgcccgccgggaggacagcgggtacttttggtttccctattggggccagggcactctcgtctccgtgagcagtgctagcactaaggggccatcagtgttccccctggccccatgcagccggagtacaagcgaatccactgccgcccttggatgcctcgtgaaggattacttccccgagcccgtgaccgtgagttggaacagcggagccttgacaagcggcgtccacacattccccgccgtcctccagtctagcgggctttacagcctcagctccgtcgtgaccgtccctagttcctccctcggaactaagacatacacttgcaacgtggatcataagccctcaaacacaaaggtcgataagcgggtcgagagcaaatacggcccaccatgcccaccttgtcccgcccccgagtttttggggggcccctctgtgttcctctttcctcctaagcctaaggacactctcatgattagccggacacccgaggtcacctgcgtcgtcgtggacgtgagccaggaggaccctgaagtgcagttcaattggtatgtggacggggtcgaggtccacaacgccaagacaaagccaagagaggagcagtttaacagtacctaccgggtcgtgagtgtgctgacagtgcttcaccaggactggctgaacgggaaggagtataagtgcaaggtgtccaacaagggcctcccctcaagcatcgagaagactatctctaaggccaaggggcagcccagagagccacaggtgtatacattgccccctagccaggaggagatgactaaaaaccaggtgtctctgacctgtctggtcaaaggcttctacccctccgatatcgctgtggagtgggagtccaacggacagccagaaaacaactacaagaccacacctcccgtcctggatagcgacggctcatttttcctatacagcaggctgaccgtggacaaatccagatggcaggagggcaacgtgttctcctgcagcgtgatgcatgaggccctgcacaaccactacactcagaagtccctgtccctgagcctgggcaaatag

SEQ ID NO: 21 - protein, 213 aa, Artificial Sequence
  Synthetic Polypeptide
NIQMTQSPSLLSASVGDRVTLSCKAGQNVNNYLAWYQQKLGEPPKVLIFNANSLQTGVPSRFSGSGSGTDFTLTISSLQPEDVATYFCQQYNSWTTFGAGTKLELKRTVAAPSVFIFPPSDEQLKSGTASVVCLLNNFYPREAKVQWKVDNALQSGNSQESVTEQDSKDSTYSLSSTLTLSKADYEKHKVYACEVTHQGLSSPVTKSFNRGEC

SEQ ID NO: 22 - DNA, 642 bp, Artificial Sequence
  Synthetic Polynucleotide
aatatccagatgacccagtccccttccctcctcagcgcttccgtgggagatagggtgacactcagttgcaaggcaggacagaacgtgaacaactacctggcctggtaccagcagaagctgggcgaacctccaaaggtccttatcttcaacgccaacagcctgcagaccggggtgccctcacggttttctgggtctgggagcggcacagactttactttgactattagctccttgcagcccgaggacgtcgccacatatttctgtcagcaatacaacagctggaccaccttcggggccggcacaaagctggagctgaaacgtacggtggctgcaccatctgtcttcatcttcccgccatctgatgagcagttgaaatctggaactgcctctgttgtgtgcctgctgaataacttctatcccagagaggccaaagtacagtggaaggtggataacgccctccaatcgggtaactcccaggagagtgtcacagagcaggacagcaaggacagcacctacagcctcagcagcaccctgacgctgagcaaagcagactacgagaaacacaaagtctacgcctgcgaagtcacccatcagggcctgagctcgcccgtcacaaagagcttcaacaggggagagtgttag

SEQ ID NO: 23 - protein, 448 aa, Artificial Sequence
  Synthetic Polypeptide
QVTLKESGPALVKPTQTLTLTCTFSGFSLSTSGTCVSWIRQPPGKALEWLATICWEDSKGYNPSLKSRLTISKDTSKNQAVLTMTNMDPVDTATYYCARREDSGYFWFPYWGQGTLVTVSSASTKGPSVFPLAPCSRSTSESTAALGCLVKDYFPEPVTVSWNSGALTSGVHTFPAVLQSSGLYSLSSVVTVPSSSLGTKTYTCNVDHKPSNTKVDKRVESKYGPPCPPCPAPEFLGGPSVFLFPPKPKDTLMISRTPEVTCVVVDVSQEDPEVQFNWYVDGVEVHNAKTKPREEQFNSTYRVVSVLTVLHQDWLNGKEYKCKVSNKGLPSSIEKTISKAKGQPREPQVYTLPPSQEEMTKNQVSLTCLVKGFYPSDIAVEWESNGQPENNYKTTPPVLDSDGSFFLYSRLTVDKSRWQEGNVFSCSVMHEALHNHYTQKSLSLSLGK

SEQ ID NO: 24 - protein, 213 aa, Artificial Sequence
  Synthetic Polypeptide
NIQMTQSPSSLSASVGDRVTITCKAGQNVNNYLAWYQQKPGKAPKVLIFNANSLQTGVPSRFSGSGSGTDFTLTISSLQPEDFATYYCQQYNSWTTFGGGTKVEIKRTVAAPSVFIFPPSDEQLKSGTASVVCLLNNFYPREAKVQWKVDNALQSGNSQESVTEQDSKDSTYSLSSTLTLSKADYEKHKVYACEVTHQGLSSPVTKSFNRGEC